European Patent Application EP 4 269 434 A1, published November 1, 2023. Title: Anti-PD-L1 Antibody and Use thereof. Applicant: Guangdong Fapon Biopharma Inc. Application EP 21909453.9. The sequence listing filed with the application follows.

SEQUENCE LISTING (42 sequences)

SEQ ID NO: 1 - protein, 290 aa, Artificial Sequence
  human PD-L1 full-length protein
MRIFAVFIFMTYWHLLNAFTVTVPKDLYVVEYGSNMTIECKFPVEKQLDLAALIVYWEMEDKNIIQFVHGEEDLKVQHSSYRQRARLLKDQLSLGNAALQITDVKLQDAGVYRCMISYGGADYKRITVKVNAPYNKINQRILVVDPVTSEHELTCQAEGYPKAEVIWTSSDHQVLSGKTTTTNSKREEKLFNVTSTLRINTTTNEIFYCTFRRLDPEENHTAELVIPELPLAHPPNERTHLVILGAILLCLGVALTFIFRLRKGRMMDVKKCGIQDTNSKKQSDTHLEET

SEQ ID NO: 2 - protein, 290 aa, Artificial Sequence
  macaque PD-L1
MRIFAVFIFTIYWHLLNAFTVTVPKDLYVVEYGSNMTIECKFPVEKQLDLTSLIVYWEMEDKNIIQFVHGEEDLKVQHSNYRQRAQLLKDQLSLGNAALRITDVKLQDAGVYRCMISYGGADYKRITVKVNAPYNKINQRILVVDPVTSEHELTCQAEGYPKAEVIWTSSDHQVLSGKTTTTNSKREEKLLNVTSTLRINTTANEIFYCIFRRLDPEENHTAELVIPELPLALPPNERTHLVILGAIFLLLGVALTFIFYLRKGRMMDMKKCGIRVTNSKKQRDTQLEET

SEQ ID NO: 3 - DNA, 342 bp, Artificial Sequence
  The nucleotide sequence of heavy chain variable region of F016-21
gaggtccagctgcagcagtctggacctgagctggtaaagcctggggcttcagtgaaaatgtcctgcaaggcttctggatacacattcactgactatgttatgcactgggtgaagcaaaaacctgggcagggccttgagtggattggatatattaatccttacaatgatggtactaagttcaatgaaaagttcaaaggcaaggccacactgacttcagacaaatcctccagcacagcctacatggagctcagcagcctgacctctgaggactctgcggtctattactgtgcaaaacaaactctggactactggggtcaaggaacctcagtcaccgtctcctca

SEQ ID NO: 4 - DNA, 336 bp, Artificial Sequence
  The nucleotide sequence of light chain variable region of F016-21
gacattgtgctcacccaatctccagcttctttggctgtgtctctagggcagagagccaccatctcctgcagagccagtgaaagtgttgaatattttggcacaactttaatgcagtggtaccaacagagaccaggacagccacccaaactcctcatctatgctgcatccaacgtagaatctggggtccctgccaggtttagtggcagtgggtctgggacagacttcagcctcaacatccatcctgtggaggaggatgatattgcaatgtatttctgtcagcaaagtaggaaggttccgtacacgttcggaggggggaccaagctggaaataaaacgg

SEQ ID NO: 5 - protein, 114 aa, Artificial Sequence
  The amino acid sequence of heavy chain variable region of F016-21
EVQLQQSGPELVKPGASVKMSCKASGYTFTDYVMHWVKQKPGQGLEWIGYINPYNDGTKFNEKFKGKATLTSDKSSSTAYMELSSLTSEDSAVYYCAKQTLDYWGQGTSVTVSS

SEQ ID NO: 6 - protein, 112 aa, Artificial Sequence
  The amino acid sequence of light chain variable region of F016-21
DIVLTQSPASLAVSLGQRATISCRASESVEYFGTTLMQWYQQRPGQPPKLLIYAASNVESGVPARFSGSGSGTDFSLNIHPVEEDDIAMYFCQQSRKVPYTFGGGTKLEIKR

SEQ ID NO: 7 - DNA, 342 bp, Artificial Sequence
  The nucleotide sequence of heavy chain variable region of F016-193
gaggtccagctgcagcagtctggacctgagctggtaaagcctggggcttcagtgaagatgtcctgcaaggcttctggatacacattcactagttatgttatgcactgggtgaagcagaagcctgggcagggccttgagtggattggatatattaatcctcacaatgatggtaataagtacaatgagaagttcaaaggcaaggccacactgacttcagacaaatcctccagctcagcctacatggagctcagcagcctgacctctgaggactctgcggtctattactgtgcaaaacagactatggactactggggtcaaggaacctcagtcaccgtctcctca

SEQ ID NO: 8 - DNA, 336 bp, Artificial Sequence
  The nucleotide sequence of light chain variable region of F016-193
gacattgtgctcacccaatctccggcttctttggctgtgtctctagggcagagagccaccctctcctgcagagccagtgaaagtgttgaattttatggcacaactttaatgcagtggttccaacagaaaccaggacagccacccaaactcctcatctatgctgcatccaacgtagaatctggggtccctgccaggtttagtggcagtgggtctgggacagacttcagcctcaacatccatcctgtggaggaggatgatattgcaatgtatttctgtcagcaaagtaggaaggttccgtacacgttcggaggggggaccaagctggaaataaaacgg

SEQ ID NO: 9 - protein, 114 aa, Artificial Sequence
  The amino acid sequence of heavy chain variable region of F016-193
EVQLQQSGPELVKPGASVKMSCKASGYTFTSYVMHWVKQKPGQGLEWIGYINPHNDGNKYNEKFKGKATLTSDKSSSSAYMELSSLTSEDSAVYYCAKQTMDYWGQGTSVTVSS

SEQ ID NO: 10 - protein, 112 aa, Artificial Sequence
  The amino acid sequence of light chain variable region of F016-193
DIVLTQSPASLAVSLGQRATLSCRASESVEFYGTTLMQWFQQKPGQPPKLLIYAASNVESGVPARFSGSGSGTDFSLNIHPVEEDDIAMYFCQQSRKVPYTFGGGTKLEIKR

SEQ ID NO: 11 - DNA, 348 bp, Artificial Sequence
  The nucleotide sequence of heavy chain variable region of F016-568
cagcttcaggagtcaggacctagcctcgtgaaaccttctcaaactctgtccctcacctgttctgtcactggcgactccatcaccagtgattactggaactggatccggaaattcccagggaataaacttgagtacatgggatacataagctacactggtagcacttactacaatccatctctcaaaagtcgaatctccatcactcgagacacatccaagaaccagtactacctgcagttgaattctgtgactactgaggacacagccacatattactgtgcaaagcaggggggatggttaaatgctatggactactggggtcaaggaacctcagtcaccgtctcctca

SEQ ID NO: 12 - DNA, 342 bp, Artificial Sequence
  The nucleotide sequence of light chain variable region of F016-568
gacattgtgatgtcacagtctccatcctccctagctgtgtcagttggagagaaggttactgtgagctgcaagtccagtcagagccttttatatagtagcaatcaaaagaactccttggcctggtaccagcagaaaccaggacagtctcctaaactgctgatttactgggcatccactagggaatctggggtccctgatcgcttcacaggcagtggatctgggacagatttcactctcaccatcagcagtgtgaaggctgaagacctggcagtttattactgtcagcaatattatggctatccgtacacgttcggaggggggaccaagctggaaataaaacgg

SEQ ID NO: 13 - protein, 116 aa, Artificial Sequence
  The amino acid sequence of heavy chain variable region of F016-568
QLQESGPSLVKPSQTLSLTCSVTGDSITSDYWNWIRKFPGNKLEYMGYISYTGSTYYNPSLKSRISITRDTSKNQYYLQLNSVTTEDTATYYCAKQGGWLNAMDYWGQGTSVTVSS

SEQ ID NO: 14 - protein, 114 aa, Artificial Sequence
  The amino acid sequence of light chain variable region of F016-568
DIVMSQSPSSLAVSVGEKVTVSCKSSQSLLYSSNQKNSLAWYQQKPGQSPKLLIYWASTRESGVPDRFTGSGSGTDFTLTISSVKAEDLAVYYCQQYYGYPYTFGGGTKLEIKR

SEQ ID NO: 15 - DNA, 357 bp, Artificial Sequence
  The nucleotide sequence of heavy chain variable region of F016-870
gaggtgcagcttcaggagtcaggacctagcctcgtgaaaccttctcagactctgtccctcacctgttctgtcactggcgactccatcaccagtggttactggaactggatccggaaattcccagggaataaacttgagtacatggggtacataagctacactggtagcacttaccagaatccatctctcaaaagtcgaatctccttcactcgagacacatccaagaaccagtactacctgcagttgagttctgtgactactgaggacacagccacatattactgtgcaagatcccgggcatggatacggacctactttgactactggggccagggcaccactctcacagtctcctca

SEQ ID NO: 16 - DNA, 327 bp, Artificial Sequence
  The nucleotide sequence of light chain variable region of F016-870
gaaattgtgctcacccagtctccagcactcatggctgcatctccaggggagaaggtcaccatcacctgcagtgtcagctcaagtataagttccagcaacttgcactggtaccagcagaagtcagaaacctcccccaaaccctggatttatggcacatccaacctggcttctggagtccctgttcgcttcagtggcagtggatctgggacctcttattctctcacaatcagcagcatggaggctgaagatgctgccacttattactgtcaacagtggagtagttacccactcacgttcggtgctgggaccaagctggagctgaaacgg

SEQ ID NO: 17 - protein, 119 aa, Artificial Sequence
  The amino acid sequence of heavy chain variable region of F016-870
EVQLQESGPSLVKPSQTLSLTCSVTGDSITSGYWNWIRKFPGNKLEYMGYISYTGSTYQNPSLKSRISFTRDTSKNQYYLQLSSVTTEDTATYYCARSRAWIRTYFDYWGQGTTLTVSS

SEQ ID NO: 18 - protein, 109 aa, Artificial Sequence
  The amino acid sequence of light chain variable region of F016-870
EIVLTQSPALMAASPGEKVTITCSVSSSISSSNLHWYQQKSETSPKPWIYGTSNLASGVPVRFSGSGSGTSYSLTISSMEAEDAATYYCQQWSSYPLTFGAGTKLELKR

SEQ ID NO: 19 - protein, 10 aa, Artificial Sequence
  HCDR1
GYTFTDYVMH

SEQ ID NO: 20 - protein, 17 aa, Artificial Sequence
  HCDR2
YINPYNDGTKFNEKFKG

SEQ ID NO: 21 - protein, 5 aa, Artificial Sequence
  HCDR3
QTLDY

SEQ ID NO: 22 - protein, 15 aa, Artificial Sequence
  LCDR1
RASESVEYFGTTLMQ

SEQ ID NO: 23 - protein, 7 aa, Artificial Sequence
  LCDR2
AASNVES

SEQ ID NO: 24 - protein, 9 aa, Artificial Sequence
  LCDR3
QQSRKVPYT

SEQ ID NO: 25 - protein, 10 aa, Artificial Sequence
  HCDR1
GYTFTSYVMH

SEQ ID NO: 26 - protein, 17 aa, Artificial Sequence
  HCDR2
YINPHNDGNKYNEKFKG

SEQ ID NO: 27 - protein, 5 aa, Artificial Sequence
  HCDR3
QTMDY

SEQ ID NO: 28 - protein, 15 aa, Artificial Sequence
  LCDR1
RASESVEFYGTTLMQ

SEQ ID NO: 29 - protein, 7 aa, Artificial Sequence
  LCDR2
AASNVES

SEQ ID NO: 30 - protein, 9 aa, Artificial Sequence
  LCDR3
QQSRKVPYT

SEQ ID NO: 31 - protein, 9 aa, Artificial Sequence
  HCDR1
GDSITSDYW

SEQ ID NO: 32 - protein, 16 aa, Artificial Sequence
  HCDR2
YISYTGSTYYNPSLKS

SEQ ID NO: 33 - protein, 10 aa, Artificial Sequence
  HCDR3
QGGWLNAMDY

SEQ ID NO: 34 - protein, 17 aa, Artificial Sequence
  LCDR1
KSSQSLLYSSNQKNSLA

SEQ ID NO: 35 - protein, 7 aa, Artificial Sequence
  LCDR2
WASTRES

SEQ ID NO: 36 - protein, 9 aa, Artificial Sequence
  LCDR3
QQYYGYPYT

SEQ ID NO: 37 - protein, 10 aa, Artificial Sequence
  HCDR1
GDSITSGYWN

SEQ ID NO: 38 - protein, 16 aa, Artificial Sequence
  HCDR2
YISYTGSTYQNPSLKS

SEQ ID NO: 39 - protein, 11 aa, Artificial Sequence
  HCDR3
SRAWIRTYFDY

SEQ ID NO: 40 - protein, 12 aa, Artificial Sequence
  LCDR1
SVSSSISSSNLH

SEQ ID NO: 41 - protein, 7 aa, Artificial Sequence
  LCDR2
GTSNLAS

SEQ ID NO: 42 - protein, 9 aa, Artificial Sequence
  LCDR3
QQWSSYPLT